European Patent Application EP 4 778 580 A1, published July 22, 2026. Title: Modified Collagen Peptides. Applicant: Fraunhofer-Gesellschaft zur Förderung, der angewandten Forschung e.V., München. Application EP. The sequence listing filed with the application follows.

SEQUENCE LISTING (25 sequences)

SEQ ID NO: 1 - protein, 15 aa, Homo sapiens
GIAGFKGEQGPKGET

SEQ ID NO: 2 - protein, 15 aa, Synthetic construct
GIAGFKGEQGPKGQT

SEQ ID NO: 3 - protein, 15 aa, Synthetic construct
GIAGFKGQQGPKGET

SEQ ID NO: 4 - protein, 15 aa, Synthetic construct
GIAGFKGQQGPKGQT

SEQ ID NO: 5 - protein, 15 aa, Synthetic construct
GIAGFKGEEGPKGET

SEQ ID NO: 6 - protein, 15 aa, Synthetic construct
GIAGFKGEEGPKGQT

SEQ ID NO: 7 - protein, 15 aa, Synthetic construct
GIAGFKGEQGPKGET

SEQ ID NO: 8 - protein, 15 aa, Synthetic construct
GIAGFKGEQGPKGQT

SEQ ID NO: 9 - protein, 11 aa, Synthetic construct
AGFKGEQGPKG

SEQ ID NO: 10 - protein, 11 aa, Synthetic construct
  VARIANT 10: note = A or R or N or D or C or Q or E or G or H or I or L or M or F or P or S or T or W or Y or V, preferably R or A or G or Q, more preferably R
AGFKGEQGPXG

SEQ ID NO: 11 - protein, 11 aa, Synthetic construct
  VARIANT 7: note = A or R or N or D or C or E or G or H or I or L or M or F or P or S or T or W or Y or V or K, preferably A or R or H or G
AGFKGEXGPKG

SEQ ID NO: 12 - protein, 11 aa, Synthetic construct
  VARIANT 6: note = A or R or N or D or C or Q or G or H or I or L or M or F or P or S or T or W or Y or V or K, preferably A or D or Q or G
AGFKGXQGPKG

SEQ ID NO: 13 - protein, 11 aa, Synthetic construct
  VARIANT 5: note = A or R or N or D or C or Q or E or H or I or L or M or F or P or S or T or W or Y or V or K, preferably A or S or V or L
AGFKXEQGPKG

SEQ ID NO: 14 - protein, 11 aa, Synthetic construct
  VARIANT 7: note = A or R or N or D or C or E or G or H or I or L or M or F or P or S or T or W or Y or V or K, preferably A or R or H or G
  VARIANT 10: note = A or R or N or D or C or Q or E or G or H or I or L or M or F or P or S or T or W or Y or V, preferably R or A or G or Q, more preferably R
AGFKGEXGPXG

SEQ ID NO: 15 - protein, 11 aa, Synthetic construct
  VARIANT 6: note = A or R or N or D or C or Q or G or H or I or L or M or F or P or S or T or W or Y or V or K, preferably A or D or Q or G
  VARIANT 10: note = A or R or N or D or C or Q or E or G or H or I or L or M or F or P or S or T or W or Y or V, preferably R or A or G or Q, more preferably R
AGFKGXQGPXG

SEQ ID NO: 16 - protein, 11 aa, Synthetic construct
  VARIANT 5: note = A or R or N or D or C or Q or E or H or I or L or M or F or P or S or T or W or Y or V or K, preferably A or S or V or L
  VARIANT 10: note = A or R or N or D or C or Q or E or G or H or I or L or M or F or P or S or T or W or Y or V, preferably R or A or G or Q, more preferably R
AGFKXEQGPXG

SEQ ID NO: 17 - protein, 11 aa, Synthetic construct
AGFKGEQGPRG

SEQ ID NO: 18 - protein, 13 aa, Synthetic construct
AGFKGEQGPKGEP

SEQ ID NO: 19 - protein, 13 aa, Synthetic construct
  VARIANT 10: note = A or R or N or D or C or Q or E or G or H or I or L or M or F or P or S or T or W or Y or V, preferably R or A or G or Q, more preferably R
AGFKGEQGPXGEP

SEQ ID NO: 20 - protein, 13 aa, Synthetic construct
AGFKGEQGPRGEP

SEQ ID NO: 21 - protein, 15 aa, Synthetic construct
GIAGFKGEQGPKGEP

SEQ ID NO: 22 - protein, 15 aa, Synthetic construct
  VARIANT 12: note = A or R or N or D or C or Q or E or G or H or I or L or M or F or P or S or T or W or Y or V, preferably R or A or G or Q, more preferably R
GIAGFKGEQGPXGEP

SEQ ID NO: 23 - protein, 15 aa, Synthetic construct
GIAGFKGEQGPRGEP

SEQ ID NO: 24 - protein, 275 aa, Homo sapiens
MKLCILLAVVAFVGLSLGIKEEHVIIQAEFYLNPDQSGEFMFDFDGDEIFHVDMAKKETVWRLEEFGRFASFEAQGALANIAVDKANLEIMTKRSNYTPITNVPPEVTVLTNSPVELREPNVLICFIDKFTPPVVNVTWLRNGKPVTTGVSETVFLPREDHLFRKFHYLPFLPSTEDVYDCRVEHWGLDEPLLKHWEFDASGGGENLYFQGGGGSLTDTLQAETDQLEDEKSALQTEIANLLKEKEKLEFILAAHGGGGSGLNDIFEAQKIEWHE

SEQ ID NO: 25 - protein, 311 aa, Synthetic construct
MKLCILLAVVAFVGLSLGSAWSHPQFEKGIAGFKGEQGPKGEPSGGGSLVPRGSGGGGSGDTRPRFLEQVKHECHFFNGTERVRFLDRYFYHQEEYVRFDSDVGEYRAVTELGRPDAEYWNSQKDLLEQKRAAVDTYCRHNYGVGESFTVQRRVYPEVTVYPAKTQPLQHHNLLVCSVNGFYPGSIEVRWFRNGQEEKTGVVSTGLIQNGDWTFQTLVMLETVPRSGEVYTCQVEHPSLTSPLTVEWRARSGGGENLYFQGGGGSRIARLEEKVKTLKAQNSELASTANMLREQVAQLKQKVMNHHHHHHH